European Patent Application EP 4 585 926 A1, published July 16, 2025. Title: Verfahren und Kit zur Reduzierung von Interferenzen in Immunoassays. Applicant: Siemens Healthcare Diagnostics Products GmbH. Application EP. The sequence listing filed with the application follows.

SEQUENCE LISTING (4 sequences)

SEQ ID NO: 1 - protein, 12 aa, Mus musculus
DTMIKGHYVMDY

SEQ ID NO: 2 - protein, 12 aa, unidentified
DTMIKGHSVFDY

SEQ ID NO: 3 - protein, 120 aa, Mus musculus
QVQLKESGPGLVAPSQSLSITCTVSGFSLTDYGVNWVRQPPGKGLEWLGMIWVDGSTDYNSALKSRLSISKDNSKSQVFLKMNSLQTDDTARYYCARDTMIKGHYVMDYWGQGTSVTVSS

SEQ ID NO: 4 - protein, 120 aa, unidentified
QVQLKESGPGLVAPSQSLSITCTVSGFSLTDYGVNWVRQPPGKGLEWLGMIWVDGSTDYNSALKSRLSISKDNSKSQVFLKMNSLQTDDTARYYCARDTMIKGHSVFDYWGQGTSVTVSS